European Patent Specification EP 3 571 196 B1, published January 4, 2023. Title: Novel Bridged Bicycloalkyl-Substituted Aminothiazoles and their Methods of Use. Applicant: Temple University - Of The Commonwealth System of Higher Education Childers, Wayne E. Abou-Gharbia, Magid A. Morton, George C. Issa, Jean-Pierre J. Zhang, Hanghang. The sequence listing filed with the application follows.

SEQUENCE LISTING (16 sequences)

SEQ ID NO: 1 - RNA, 21 nt, Artificial sequence
  chemically synthesized
ggauugcccugagcuaauuuu

SEQ ID NO: 2 - DNA, 6 bp, Artificial sequence
  chemically synthesized
cccggg

SEQ ID NO: 3 - protein, 23 aa, Artificial sequence
  chemically synthesized
KIPDPDSDDVSEVDARHIIENAK

SEQ ID NO: 4 - protein, 20 aa, Artificial sequence
  chemically synthesized
YKDSSSGRQLSEVFIQLPSR

SEQ ID NO: 5 - DNA, 23 bp, Artificial sequence
  chemically synthesized
gaattcagtgccactaagcagac

SEQ ID NO: 6 - DNA, 23 bp, Artificial sequence
  chemically synthesized
tcggtatatccaagacatgatcc

SEQ ID NO: 7 - DNA, 24 bp, Artificial sequence
  chemically synthesized
atatccctcaccacgatcctaata

SEQ ID NO: 8 - DNA, 24 bp, Artificial sequence
  chemically synthesized
ccctctgtagtgcaaagactgata

SEQ ID NO: 9 - DNA, 23 bp, Artificial sequence
  chemically synthesized
tcttggagtcctcactcaaactc

SEQ ID NO: 10 - DNA, 23 bp, Artificial sequence
  chemically synthesized
actgctgcaactacccttaaaca

SEQ ID NO: 11 - DNA, 23 bp, Artificial sequence
  chemically synthesized
caggaaactaactttcagccaga

SEQ ID NO: 12 - DNA, 23 bp, Artificial sequence
  chemically synthesized
taaagagggcatggagtaattga

SEQ ID NO: 13 - DNA, 20 bp, Artificial sequence
  chemically synthesized
tctcacaatcctggaggctg

SEQ ID NO: 14 - DNA, 20 bp, Artificial sequence
  chemically synthesized
gaccaagaagcaagccctca

SEQ ID NO: 15 - DNA, 19 bp, Artificial sequence
  chemically synthesized
cagacagacactggcaaca

SEQ ID NO: 16 - DNA, 19 bp, Artificial sequence
  chemically synthesized
acatctcccccttctcctt